European Patent Specification EP 3 483 289 B1, published June 11, 2025. Title: COMPOSITIONS AND METHODS FOR DETERMINING RESISTANCE TO INHIBITORS OF VIRUS ENTRY USING RECOMBINANT VIRUS ASSAYS. Applicant: Petropoulos, Christos J. Application EP 11161793.2. The sequence listing filed with the application follows.

SEQUENCE LISTING (10 sequences)

SEQ ID NO: 1 - DNA, 26 bp, Artificial sequence
  Synthetic construct
ggagcatttacaagcagcaacacagc

SEQ ID NO: 2 - DNA, 21 bp, Artificial sequence
  Synthetic construct
ttccagtcavacctcaggtac

SEQ ID NO: 3 - DNA, 19 bp, Artificial sequence
  Synthetic construct
agaccaatgacttayaagg

SEQ ID NO: 4 - DNA, 35 bp, Artificial sequence
  Synthetic construct
gggctcgagaccggtcagtggcaatgagagtgaag

SEQ ID NO: 5 - DNA, 37 bp, Artificial sequence
  Synthetic construct
gggctcgagaccggtgagcagaagacagtggcaatga

SEQ ID NO: 6 - DNA, 36 bp, Artificial sequence
  Synthetic construct
gggctcgagaccggtgagcagaagacagtggcaatg

SEQ ID NO: 7 - DNA, 35 bp, Artificial sequence
  Synthetic construct
gggtctagaacgcgttgccacccatcttatagcaa

SEQ ID NO: 8 - DNA, 38 bp, Artificial sequence
  Synthetic construct
gggtctagaacgcgtccacttgccacccatbttatagc

SEQ ID NO: 9 - DNA, 33 bp, Artificial sequence
  Synthetic construct
gggtctagaacgcgtccacttgccacccatbtt

SEQ ID NO: 10 - DNA, 38 bp, Artificial sequence
  Synthetic construct
gatggtctaagacgctgttcaatatccctgcctaactc